European Patent Specification EP 3 515 476 B1, published May 22, 2024. Title: A NOVEL COMPLEX COMPRISING A CELL PENETRATING PEPTIDE, A CARGO AND A TLR PEPTIDE AGONIST FOR TREATMENT OF COLORECTAL CANCER. Applicant: Amal Therapeutics SA, Geneva, Switzerland. The sequence listing filed with the application follows.

SEQUENCE LISTING (98 sequences)

SEQ ID NO: 1 - protein, 16 aa, Artificial Sequence
  CPP: Penetratin
RQIKIYFQNRRMKWKK

SEQ ID NO: 2 - protein, 11 aa, Artificial Sequence
  CPP: TAT minimal domain
YGRKKRRQRRR

SEQ ID NO: 3 - protein, 245 aa, Artificial Sequence
  ZEBRA amino acid sequence (natural sequence from Epstein - Barr virus (EBV)) (YP_401673)
MMDPNSTSEDVKFTPDPYQVPFVQAFDQATRVYQDLGGPSQAPLPCVLWPVLPEPLPQGQLTAYHVSTAPTGSWFSAPQPAPENAYQAYAAPQLFPVSDITQNQQTNQAGGEAPQPGDNSTVQTAAAVVFACPGANQGQQLADIGVPQPAPVAAPARRTRKPQQPESLEECDSELEIKRYKNRVASRKCRAKFKQLLQHYREVAAAKSSENDRLRLLLKQMCPSLDVDSIIPRTPDVLHEDLLNF

SEQ ID NO: 4 - protein, 45 aa, Artificial Sequence
  CPP1 (Z11)
KRYKNRVASRKCRAKFKQLLQHYREVAAAKSSENDRLRLLLKQMC

SEQ ID NO: 5 - protein, 42 aa, Artificial Sequence
  CPP2 (Z12)
KRYKNRVASRKCRAKFKQLLQHYREVAAAKSSENDRLRLLLK

SEQ ID NO: 6 - protein, 42 aa, Artificial Sequence
  CPP3 (Z13)
KRYKNRVASRKSRAKFKQLLQHYREVAAAKSSENDRLRLLLK

SEQ ID NO: 7 - protein, 30 aa, Artificial Sequence
  CPP4 (Z14)
KRYKNRVASRKSRAKFKQLLQHYREVAAAK

SEQ ID NO: 8 - protein, 17 aa, Artificial Sequence
  CPP5 (Z15)
KRYKNRVASRKSRAKFK

SEQ ID NO: 9 - protein, 15 aa, Artificial Sequence
  CPP6 (Z16)
QHYREVAAAKSSEND

SEQ ID NO: 10 - protein, 13 aa, Artificial Sequence
  CPP7 (Z17)
QLLQHYREVAAAK

SEQ ID NO: 11 - protein, 19 aa, Artificial Sequence
  CPP8 (Z18)
REVAAAKSSENDRLRLLLK

SEQ ID NO: 12 - protein, 8 aa, Artificial Sequence
  CPP9 (Z19)
KRYKNRVA

SEQ ID NO: 13 - protein, 11 aa, Artificial Sequence
  CPP10 (Z20)
VASRKSRAKFK

SEQ ID NO: 14 - protein, 85 aa, Artificial Sequence
  MAD5 cargo
ESLKISQAVHAAHAEINEAGREVVGVGALKVPRNQDWLGVPRFAKFASFEAQGALANIAVDKANLDVEQLESIINFEKLTEWTGS

SEQ ID NO: 15 - protein, 35 aa, Artificial Sequence
  TLR2 peptide agonist Anaxa
STVHEILCKLSLEGDHSTPPSAYGSVKPYTNFDAE

SEQ ID NO: 16 - protein, 4 aa, Artificial Sequence
  enterokinase target site
DDDK

SEQ ID NO: 17 - protein, 5 aa, Artificial Sequence
  factor Xa target site
IEDGR

SEQ ID NO: 18 - protein, 6 aa, Artificial Sequence
  thrombin target site
LVPRGS

SEQ ID NO: 19 - protein, 7 aa, Artificial Sequence
  protease TEV target site
ENLYFQG

SEQ ID NO: 20 - protein, 8 aa, Artificial Sequence
  PreScission protease target site
LEVLFQGP

SEQ ID NO: 21 - protein, 4 aa, Artificial Sequence
  furin target site
  MISC_FEATURE (2)..(2): X may be any amino acid
  MISC_FEATURE (3)..(3): X is R or K
RXXR

SEQ ID NO: 22 - protein, 5 aa, Artificial Sequence
  peptidic linker
GGGGG

SEQ ID NO: 23 - protein, 4 aa, Artificial Sequence
  peptidic linker
GGGG

SEQ ID NO: 24 - protein, 4 aa, Artificial Sequence
  peptidic linker
EQLE

SEQ ID NO: 25 - protein, 4 aa, Artificial Sequence
  peptidic linker
TEWT

SEQ ID NO: 26 - protein, 224 aa, Artificial Sequence
  EDAZ13Mad5
MHHHHHHNIDRPKGLAFTDVDVDSIKIAWESPQGQVSRYRVTYSSPEDGIRELFPAPDGEDDTAELQGLRPGSEYTVSVVALHDDMESQPLIGIQSTKRYKNRVASRKSRAKFKQLLQHYREVAAAKSSENDRLRLLLKESLKISQAVHAAHAEINEAGREVVGVGALKVPRNQDWLGVPRFAKFASFEAQGALANIAVDKANLDVEQLESIINFEKLTEWTGS

SEQ ID NO: 27 - protein, 169 aa, Artificial Sequence
  AnaxaZ13Mad5
MHHHHHHSTVHEILCKLSLEGDHSTPPSAYGSVKPYTNFDAEKRYKNRVASRKSRAKFKQLLQHYREVAAAKSSENDRLRLLLKESLKISQAVHAAHAEINEAGREVVGVGALKVPRNQDWLGVPRFAKFASFEAQGALANIAVDKANLDVEQLESIINFEKLTEWTGS

SEQ ID NO: 28 - protein, 169 aa, Artificial Sequence
  Z13Mad5Anaxa
MHHHHHHKRYKNRVASRKSRAKFKQLLQHYREVAAAKSSENDRLRLLLKESLKISQAVHAAHAEINEAGREVVGVGALKVPRNQDWLGVPRFAKFASFEAQGALANIAVDKANLDVEQLESIINFEKLTEWTGSSTVHEILCKLSLEGDHSTPPSAYGSVKPYTNFDAE

SEQ ID NO: 29 - protein, 134 aa, Artificial Sequence
  Z13Mad5
MHHHHHHKRYKNRVASRKSRAKFKQLLQHYREVAAAKSSENDRLRLLLKESLKISQAVHAAHAEINEAGREVVGVGALKVPRNQDWLGVPRFAKFASFEAQGALANIAVDKANLDVEQLESIINFEKLTEWTGS

SEQ ID NO: 30 - protein, 92 aa, Artificial Sequence
  Mad5
MHHHHHHESLKISQAVHAAHAEINEAGREVVGVGALKVPRNQDWLGVPRFAKFASFEAQGALANIAVDKANLDVEQLESIINFEKLTEWTGS

SEQ ID NO: 31 - protein, 182 aa, Artificial Sequence
  EdaMad5
MHHHHHHNIDRPKGLAFTDVDVDSIKIAWESPQGQVSRYRVTYSSPEDGIRELFPAPDGEDDTAELQGLRPGSEYTVSVVALHDDMESQPLIGIQSTESLKISQAVHAAHAEINEAGREVVGVGALKVPRNQDWLGVPRFAKFASFEAQGALANIAVDKANLDVEQLESIINFEKLTEWTGS

SEQ ID NO: 32 - protein, 127 aa, Artificial Sequence
  Mad5Anaxa
MHHHHHHESLKISQAVHAAHAEINEAGREVVGVGALKVPRNQDWLGVPRFAKFASFEAQGALANIAVDKANLDVEQLESIINFEKLTEWTGSSTVHEILCKLSLEGDHSTPPSAYGSVKPYTNFDAE

SEQ ID NO: 33 - protein, 157 aa, Artificial Sequence
  Z14Mad5Anaxa
MHHHHHHKRYKNRVASRKSRAKFKQLLQHYREVAAAKESLKISQAVHAAHAEINEAGREVVGVGALKVPRNQDWLGVPRFAKFASFEAQGALANIAVDKANLDVEQLESIINFEKLTEWTGSSTVHEILCKLSLEGDHSTPPSAYGSVKPYTNFDAE

SEQ ID NO: 34 - protein, 146 aa, Artificial Sequence
  Z18Mad5Anaxa
MHHHHHHREVAAAKSSENDRLRLLLKESLKISQAVHAAHAEINEAGREVVGVGALKVPRNQDWLGVPRFAKFASFEAQGALANIAVDKANLDVEQLESIINFEKLTEWTGSSTVHEILCKLSLEGDHSTPPSAYGSVKPYTNFDAE

SEQ ID NO: 35 - protein, 8 aa, Artificial Sequence
  SIINFEKL OVACD8
SIINFEKL

SEQ ID NO: 36 - protein, 17 aa, Artificial Sequence
  OVACD4 peptide
ISQAVHAAHAEINEAGR

SEQ ID NO: 37 - protein, 212 aa, Artificial Sequence
  EDAZ14Mad5
MHHHHHHNIDRPKGLAFTDVDVDSIKIAWESPQGQVSRYRVTYSSPEDGIRELFPAPDGEDDTAELQGLRPGSEYTVSVVALHDDMESQPLIGIQSTKRYKNRVASRKSRAKFKQLLQHYREVAAAKESLKISQAVHAAHAEINEAGREVVGVGALKVPRNQDWLGVPRFAKFASFEAQGALANIAVDKANLDVEQLESIINFEKLTEWTGS

SEQ ID NO: 38 - protein, 201 aa, Artificial Sequence
  EDAZ18Mad5
MHHHHHHNIDRPKGLAFTDVDVDSIKIAWESPQGQVSRYRVTYSSPEDGIRELFPAPDGEDDTAELQGLRPGSEYTVSVVALHDDMESQPLIGIQSTREVAAAKSSENDRLRLLLKESLKISQAVHAAHAEINEAGREVVGVGALKVPRNQDWLGVPRFAKFASFEAQGALANIAVDKANLDVEQLESIINFEKLTEWTGS

SEQ ID NO: 39 - protein, 116 aa, Artificial Sequence
  Z13Mad8Anaxa
KRYKNRVASRKSRAKFKQLLQHYREVAAAKSSENDRLRLLLKVTYHSPSYAYHQFERRAILNRLVQFIKDRISVVQALVLTSTVHEILCKLSLEGDHSTPPSAYGSVKPYTNFDAE

SEQ ID NO: 40 - protein, 110 aa, Artificial Sequence
  Z13Mad11Anaxa
KRYKNRVASRKSRAKFKQLLQHYREVAAAKSSENDRLRLLLKNYRIATFKNWPFLEDCAMEELTVSEFLKLDRQRSTVHEILCKLSLEGDHSTPPSAYGSVKPYTNFDAE

SEQ ID NO: 41 - protein, 94 aa, Artificial Sequence
  Z13Mad9Anaxa
KRYKNRVASRKSRAKFKQLLQHYREVAAAKSSENDRLRLLLKHLELASMTNMELMSSIVSTVHEILCKLSLEGDHSTPPSAYGSVKPYTNFDAE

SEQ ID NO: 42 - protein, 17 aa, Artificial Sequence
  Mad9
HLELASMTNMELMSSIV

SEQ ID NO: 43 - protein, 20 aa, Artificial Sequence
  Mad8
VTYHSPSYAYHQFERRAILN

SEQ ID NO: 44 - protein, 33 aa, Artificial Sequence
  Mad11
NYRIATFKNWPFLEDCAMEELTVSEFLKLDRQR

SEQ ID NO: 45 - protein, 90 aa, Artificial Sequence
  EDA
NIDRPKGLAFTDVDVDSIKIAWESPQGQVSRYRVTYSSPEDGIRELFPAPDGEDDTAELQGLRPGSEYTVSVVALHDDMESQPLIGIQST

SEQ ID NO: 46 - protein, 115 aa, Artificial Sequence
  TatFMad5Anaxa
RKKRRQRRRRVKRISQAVHAAHAEINEAGRRVKRKVPRNQDWLRVKRASFEAQGALANIAVDKARVKRSIINFEKLRVKRSTVHEILCKLSLEGDHSTPPSAYGSVKPYTNFDAE

SEQ ID NO: 47 - protein, 314 aa, Artificial Sequence
  EpCAM
MAPPQVLAFGLLLAAATATFAAAQEECVCENYKLAVNCFVNNNRQCQCTSVGAQNTVICSKLAAKCLVMKAEMNGSKLGRRAKPEGALQNNDGLYDPDCDESGLFKAKQCNGTSMCWCVNTAGVRRTDKDTEITCSERVRTYWIIIELKHKAREKPYDSKSLRTALQKEITTRYQLDPKFITSILYENNVITIDLVQNSSQKTQNDVDIADVAYYFEKDVKGESLFHSKKMDLTVNGEQLDLDPGQTLIYYVDEKAPEFSMQGLKAGVIAVIVVVVIAVVAGIVVLVISRKKRMAKYEKAEIKEMGEMHRELNA

SEQ ID NO: 48 - protein, 9 aa, Artificial Sequence
  EpCAM epitope
GLKAGVIAV

SEQ ID NO: 49 - protein, 1255 aa, Artificial Sequence
  MUC-1
MTPGTQSPFFLLLLLTVLTVVTGSGHASSTPGGEKETSATQRSSVPSSTEKNAVSMTSSVLSSHSPGSGSSTTQGQDVTLAPATEPASGSAATWGQDVTSVPVTRPALGSTTPPAHDVTSAPDNKPAPGSTAPPAHGVTSAPDTRPAPGSTAPPAHGVTSAPDTRPAPGSTAPPAHGVTSAPDTRPAPGSTAPPAHGVTSAPDTRPAPGSTAPPAHGVTSAPDTRPAPGSTAPPAHGVTSAPDTRPAPGSTAPPAHGVTSAPDTRPAPGSTAPPAHGVTSAPDTRPAPGSTAPPAHGVTSAPDTRPAPGSTAPPAHGVTSAPDTRPAPGSTAPPAHGVTSAPDTRPAPGSTAPPAHGVTSAPDTRPAPGSTAPPAHGVTSAPDTRPAPGSTAPPAHGVTSAPDTRPAPGSTAPPAHGVTSAPDTRPAPGSTAPPAHGVTSAPDTRPAPGSTAPPAHGVTSAPDTRPAPGSTAPPAHGVTSAPDTRPAPGSTAPPAHGVTSAPDTRPAPGSTAPPAHGVTSAPDTRPAPGSTAPPAHGVTSAPDTRPAPGSTAPPAHGVTSAPDTRPAPGSTAPPAHGVTSAPDTRPAPGSTAPPAHGVTSAPDTRPAPGSTAPPAHGVTSAPDTRPAPGSTAPPAHGVTSAPDTRPAPGSTAPPAHGVTSAPDTRPAPGSTAPPAHGVTSAPDTRPAPGSTAPPAHGVTSAPDTRPAPGSTAPPAHGVTSAPDTRPAPGSTAPPAHGVTSAPDTRPAPGSTAPPAHGVTSAPDTRPAPGSTAPPAHGVTSAPDTRPAPGSTAPPAHGVTSAPDTRPAPGSTAPPAHGVTSAPDTRPAPGSTAPPAHGVTSAPDTRPAPGSTAPPAHGVTSAPDTRPAPGSTAPPAHGVTSAPDTRPAPGSTAPPAHGVTSAPDTRPAPGSTAPPAHGVTSAPDTRPAPGSTAPPAHGVTSAPDNRPALGSTAPPVHNVTSASGSASGSASTLVHNGTSARATTTPASKSTPFSIPSHHSDTPTTLASHSTKTDASSTHHSSVPPLTSSNHSTSPQLSTGVSFFFLSFHISNLQFNSSLEDPSTDYYQELQRDISEMFLQIYKQGGFLGLSNIKFRPGSVVVQLTLAFREGTINVHDVETQFNQYKTEAASRYNLTISDVSVSDVPFPFSAQSGAGVPGWGIALLVLVCVLVALAIVYLIALAVCQCRRKNYGQLDIFPARDTYHPMSEYPTYHTHGRYVPPSSTDRSPYEKVSAGNGGSSLSYTNPAVAATSANL

SEQ ID NO: 50 - protein, 9 aa, Artificial Sequence
  MUC-1 epitope
GSTAPPVHN

SEQ ID NO: 51 - protein, 10 aa, Artificial Sequence
  MUC-1 epitope
TAPPAHGVTS

SEQ ID NO: 52 - protein, 142 aa, Artificial Sequence
  survivin
MGAPTLPPAWQPFLKDHRISTFKNWPFLEGCACTPERMAEAGFIHCPTENEPDLAQCFFCFKELEGWEPDDDPIEEHKKHSSGCAFLSVKKQFEELTLGEFLKLDRERAKNKIAKETNNKKKEFEETAKKVRRAIEQLAAMD

SEQ ID NO: 53 - protein, 10 aa, Artificial Sequence
  survivin epitope
RISTFKNWPF

SEQ ID NO: 54 - protein, 701 aa, Artificial Sequence
  CEA
MESPSAPPHRWCIPWQRLLLTASLLTFWNPPTTAKLTIESTPFNVAEGKEVLLLVHNLPQHLFGYSWYKGERVDGNRQIIGYVIGTQQATPGPAYSGREIIYPNASLLIQNIIQNDTGFYTLHVIKSDLVNEEATGQFRVYPELPKPSISSNNSKPVEDKDAVAFTCEPETQDATYLWWVNNQSLPVSPRLQLSNGNRTLTLFNVTRNDTASYKCETQNPVSARRSDSVILNVLYGPDAPTISPLNTSYRSGENLNLSCHAASNPPAQYSWFVNGTFQQSTQELFIPNITVNNSGSYTCQAHNSDTGLNRTTVTTITVYAEPPKPFITSNNSNPVEDEDAVALTCEPEIQNTTYLWWVNNQSLPVSPRLQLSNDNRTLTLLSVTRNDVGPYECGIQNKLSVDHSDPVILNVLYGPDDPTISPSYTYYRPGVNLSLSCHAASNPPAQYSWLIDGNIQQHTQELFISNITEKNSGLYTCQANNSASGHSRTTVKTITVSAELPKPSISSNNSKPVEDKDAVAFTCEPEAQNTTYLWWVNGQSLPVSPRLQLSNGNRTLTLFNVTRNDARAYVCGIQNSVSANRSDPVTLDVLYGPDTPIISPPDSSYLSGANLNLSCHSASNPSPQYSWRINGIPQQHTQVLFIAKITPNNNGTYACFVSNLATGRNNSIVKSITVSASGTSPGLSAGATVGIMIGVLVGVAL

SEQ ID NO: 55 - protein, 10 aa, Artificial Sequence
  CEA epitope
YLSGANLNLS

SEQ ID NO: 56 - protein, 10 aa, Artificial Sequence
  CEA epitope
SWRINGIPQQ

SEQ ID NO: 57 - protein, 189 aa, Artificial Sequence [sequence omitted]

SEQ ID NO: 58 - protein, 9 aa, Artificial Sequence
  Kirsten Ras epitope
VVVGAGGVG

SEQ ID NO: 59 - protein, 314 aa, Artificial Sequence
  MAGE-A3
MPLEQRSQHCKPEEGLEARGEALGLVGAQAPATEEQEAASSSSTLVEVTLGEVPAAESPDPPQSPQGASSLPTTMNYPLWSQSYEDSSNQEEEGPSTFPDLESEFQAALSRKVAELVHFLLLKYRAREPVTKAEMLGSVVGNWQYFFPVIFSKAFSSLQLVFGIELMEVDPIGHLYIFATCLGLSYDGLLGDNQIMPKAGLLIIVLAIIAREGDCAPEEKIWEELSVLEVFEGREDSILGDPKKLLTQHFVQENYLEYRQVPGSDPACYEFLWGPRALVETSYVKVLHHMVKISGGPHISYPPLHEWVLREGEE

SEQ ID NO: 60 - protein, 9 aa, Artificial Sequence
  MAGE-A3 epitope
KVAELVHFL

SEQ ID NO: 61 - protein, 380 aa, Artificial Sequence
  IL13Ralpha2
MAFVCLAIGCLYTFLISTTFGCTSSSDTEIKVNPPQDFEIVDPGYLGYLYLQWQPPLSLDHFKECTVEYELKYRNIGSETWKTIITKNLHYKDGFDLNKGIEAKIHTLLPWQCTNGSEVQSSWAETTYWISPQGIPETKVQDMDCVYYNWQYLLCSWKPGIGVLLDTNYNLFYWYEGLDHALQCVDYIKADGQNIGCRFPYLEASDYKDFYICVNGSSENKPIRSSYFTFQLQNIVKPLPPVYLTFTRESSCEIKLKWSIPLGPIPARCFDYEIEIREDDTTLVTATVENETYTLKTTNETRQLCFVVRSKVNIYCSDDGIWSEWSDKQCWEGEDLSKKTLLRFWLPFGFILILVIFVTGLLLRKPNTYPKMIPEFFCDT

SEQ ID NO: 62 - protein, 7 aa, Artificial Sequence
  IL13Ralpha2 epitope
LPFGFIL

SEQ ID NO: 63 - protein, 50 aa, Artificial Sequence
  Mad12
LFRAAQLANDVVLQIMEHLELASMTNMELMSSIVVISASIIVFNLLELEG

SEQ ID NO: 64 - protein, 14 aa, Artificial Sequence
  gp70CD4 peptide
LVQFIKDRISVVQA

SEQ ID NO: 65 - protein, 9 aa, Artificial Sequence
  gp70CD8 peptide
SPSYVYHQF

SEQ ID NO: 66 - protein, 9 aa, Artificial Sequence
  adpgk peptide
ASMTNMELM

SEQ ID NO: 67 - protein, 8 aa, Artificial Sequence
  survivin20-28
ATKNWPFL

SEQ ID NO: 68 - protein, 8 aa, Artificial Sequence
  survivin97-104
TVSEFLKL

SEQ ID NO: 69 - protein, 127 aa, Artificial Sequence
  Z13Mad12Anaxa
KRYKNRVASRKSRAKFKQLLQHYREVAAAKSSENDRLRLLLKLFRAAQLANDVVLQIMEHLELASMTNMELMSSIVVISASIIVFNLLELEGSTVHEILCKLSLEGDHSTPPSAYGSVKPYTNFDAE

SEQ ID NO: 70 - protein, 1255 aa, Artificial Sequence [sequence omitted]

SEQ ID NO: 71 - protein, 35 aa, Artificial Sequence
  TLR peptide agonist "Anaxa" sequence variant
STVHEILSKLSLEGDHSTPPSAYGSVKPYTNFDAE

SEQ ID NO: 72 - protein, 118 aa, Artificial Sequence
  ATP110
KRYKNRVASRKSRAKFKQLLQHYREVAAAKSSENDRLRLLLKAPPQVLAFGLLLAAATAYVDEKAPEFSMQGLKAGVIAVIVVSTVHEILCKLSLEGDHSTPPSAYGSVKPYTNFDAE

SEQ ID NO: 73 - protein, 331 aa, Artificial Sequence
  ATP111
KRYKNRVASRKSRAKFKQLLQHYREVAAAKSSENDRLRLLLKRTLTLFNVTRNDARAYVSGIQNSVSANRSDPVTPDSSYLSGANLNLSSHSASPQYSWRINGIPQQHTQVLFIAKITPNNNGTYACFVSNLATGRNNSIVKSITVSASGTSPGLSAGATVGIMIGVLVGVALILGDPKKLLTQHFVQENYLEYRQVPGSDPASYEFLWGPRALVETSYVKVALSRKVAELVHFLLLKYRAREPVTKAEMLGSVVAPPQVLAFGLLLAAATAYVDEKAPEFSMQGLKAGVIAVIVVSTVHEILCKLSLEGDHSTPPSAYGSVKPYTNFDAE

SEQ ID NO: 74 - protein, 313 aa, Artificial Sequence
  ATP112
KRYKNRVASRKSRAKFKQLLQHYREVAAAKSSENDRLRLLLKRTLTLFNVTRNDARAYVSGIQNSVSANRSDPVTPDSSYLSGANLNLSSHSASPQYSWRINGIPQQHTQVLFIAKITPNNNGTYACFVSNLATGRNNSIVKSITVSASGTSPGLSLGDPKKLLTQHFVQENYLEYRQVPGSDPASYEFLWGPRALVETSYVKVALSRKVAELVHFLLLKYRAREPVTKAEMLGSVVAPPQVLAFGLLLAAATAYVDEKAPEFSMQGLKAGVIAVIVVSTVHEILCKLSLEGDHSTPPSAYGSVKPYTNFDAE

SEQ ID NO: 75 - protein, 366 aa, Artificial Sequence
  ATP113
KRYKNRVASRKSRAKFKQLLQHYREVAAAKSSENDRLRLLLKRTLTLFNVTRNDARAYVSGIQNSVSANRSDPVTPDSSYLSGANLNLSSHSASPQYSWRINGIPQQHTQVLFIAKITPNNNGTYACFVSNLATGRNNSIVKSITVSASGTSPGLSLGDPKKLLTQHFVQENYLEYRQVPGSDPASYEFLWGPRALVETSYVKVALSRKVAELVHFLLLKYRAREPVTKAEMLGSVVAPPQVLAFGLLLAAATAYVDEKAPEFSMQGLKAGVIAVIVVAPGSTAPPAHGVTSAPDTRPAPGSTAPPAHGVTSAPDRPALGSTAPPVHNVTSSTVHEILCKLSLEGDHSTPPSAYGSVKPYTNFDAE

SEQ ID NO: 76 - protein, 335 aa, Artificial Sequence
  ATP114
KRYKNRVASRKSRAKFKQLLQHYREVAAAKSSENDRLRLLLKRTLTLFNVTRNDARAYVSGIQNSVSANRSDPVTPDSSYLSGANLNLSSHSASPQYSWRINGIPQQHTQVLFIAKITPNNNGTYACFVSNLATGRNNSIVKSITVSASGTSPGLSAPTLPPAWQPFLKDHRISTFKNWPFLEGSAVKKQFEELTLGEFLKLDRERAPPQVLAFGLLLAAATAYVDEKAPEFSMQGLKAGVIAVIVVAPGSTAPPAHGVTSAPDTRPAPGSTAPPAHGVTSAPDRPALGSTAPPVHNVTSSTVHEILCKLSLEGDHSTPPSAYGSVKPYTNFDAE

SEQ ID NO: 77 - protein, 303 aa, Artificial Sequence
  ATP115
KRYKNRVASRKSRAKFKQLLQHYREVAAAKSSENDRLRLLLKRTLTLFNVTRNDARAYVSGIQNSVSANRSDPVTPDSSYLSGANLNLSSHSASPQYSWRINGIPQQHTQVLFIAKITPNNNGTYACFVSNLATGRNNSIVKSITVSASGTSPGLSEYKLVVVGAVGVGKSALTAPPQVLAFGLLLAAATAYVDEKAPEFSMQGLKAGVIAVIVVAPGSTAPPAHGVTSAPDTRPAPGSTAPPAHGVTSAPDRPALGSTAPPVHNVTSSTVHEILCKLSLEGDHSTPPSAYGSVKPYTNFDAE

SEQ ID NO: 78 - protein, 363 aa, Artificial Sequence
  ATP116
KRYKNRVASRKSRAKFKQLLQHYREVAAAKSSENDRLRLLLKRTLTLFNVTRNDARAYVSGIQNSVSANRSDPVTPDSSYLSGANLNLSSHSASPQYSWRINGIPQQHTQVLFIAKITPNNNGTYACFVSNLATGRNNSIVKSITVSASGTSPGLSAPTLPPAWQPFLKDHRISTFKNWPFLEGSAVKKQFEELTLGEFLKLDRERAPPQVLAFGLLLAAATAYVDEKAPEFSMQGLKAGVIAVIVVLGDPKKLLTQHFVQENYLEYRQVPGSDPASYEFLWGPRALVETSYVKVALSRKVAELVHFLLLKYRAREPVTKAEMLGSVVSTVHEILCKLSLEGDHSTPPSAYGSVKPYTNFDAE

SEQ ID NO: 79 - protein, 285 aa, Artificial Sequence
  ATP117
KRYKNRVASRKSRAKFKQLLQHYREVAAAKSSENDRLRLLLKRTLTLFNVTRNDARAYVSGIQNSVSANRSDPVTPDSSYLSGANLNLSSHSASPQYSWRINGIPQQHTQVLFIAKITPNNNGTYACFVSNLATGRNNSIVKSITVSASGTSPGLSAPPQVLAFGLLLAAATAYVDEKAPEFSMQGLKAGVIAVIVVAPGSTAPPAHGVTSAPDTRPAPGSTAPPAHGVTSAPDRPALGSTAPPVHNVTSSTVHEILCKLSLEGDHSTPPSAYGSVKPYTNFDAE

SEQ ID NO: 80 - protein, 232 aa, Artificial Sequence
  ATP118
KRYKNRVASRKSRAKFKQLLQHYREVAAAKSSENDRLRLLLKRTLTLFNVTRNDARAYVSGIQNSVSANRSDPVTPDSSYLSGANLNLSSHSASPQYSWRINGIPQQHTQVLFIAKITPNNNGTYACFVSNLATGRNNSIVKSITVSASGTSPGLSAPPQVLAFGLLLAAATAYVDEKAPEFSMQGLKAGVIAVIVVSTVHEILCKLSLEGDHSTPPSAYGSVKPYTNFDAE

SEQ ID NO: 81 - protein, 261 aa, Artificial Sequence
  ATP119
KRYKNRVASRKSRAKFKQLLQHYREVAAAKSSENDRLRLLLKLGDPKKLLTQHFVQENYLEYRQVPGSDPASYEFLWGPRALVETSYVKVALSRKVAELVHFLLLKYRAREPVTKAEMLGSVVAPTLPPAWQPFLKDHRISTFKNWPFLEGSAVKKQFEELTLGEFLKLDRERAPGSTAPPAHGVTSAPDTRPAPGSTAPPAHGVTSAPDRPALGSTAPPVHNVTSSTVHEILCKLSLEGDHSTPPSAYGSVKPYTNFDAE

SEQ ID NO: 82 - protein, 191 aa, Artificial Sequence
  ATP120
KRYKNRVASRKSRAKFKQLLQHYREVAAAKSSENDRLRLLLKRTLTLFNVTRNDARAYVSGIQNSVSANRSDPVTPDSSYLSGANLNLSSHSASPQYSWRINGIPQQHTQVLFIAKITPNNNGTYACFVSNLATGRNNSIVKSITVSASGTSPGLSSTVHEILCKLSLEGDHSTPPSAYGSVKPYTNFDAE

SEQ ID NO: 83 - protein, 311 aa, Artificial Sequence
  ATP121
KRYKNRVASRKSRAKFKQLLQHYREVAAAKSSENDRLRLLLKNRTLTLFNVTRNDARAYVSGIQNSVSANRSDPVTLDVLPDSSYLSGANLNLSSHSASPQYSWRINGIPQQHTQVLFIAKITPNNNGTYACFVSNLATGRNNSIVKSITVSASGTSPGLSAGATVGIMIGVLVGVALIAPGSTAPPAHGVTSAPDTRPAPGSTAPPAHGVTSAPDRPALGSTAPPVHNVTSAPPQVLAFGLLLAAATALIYYVDEKAPEFSMQGLKAGVIAVIVVSTVHEILCKLSLEGDHSTPPSAYGSVKPYTNFDAE

SEQ ID NO: 84 - protein, 294 aa, Artificial Sequence
  ATP122
KRYKNRVASRKSRAKFKQLLQHYREVAAAKSSENDRLRLLLKNRTLTLFNVTRNDARAYVSGIQNSVSANRSDPVTLDVLPDSSYLSGANLNLSSHSASPQYSWRINGIPQQHTQVLFIAKITPNNNGTYACFVSNLATGRNNSIVKSITVSASGTSPGLSAAPGSTAPPAHGVTSAPDTRPAPGSTAPPAHGVTSAPDRPALGSTAPPVHNVTSAPPQVLAFGLLLAAATALIYYVDEKAPEFSMQGLKAGVIAVIVVSTVHEILCKLSLEGDHSTPPSAYGSVKPYTNFDAE

SEQ ID NO: 85 - protein, 294 aa, Artificial Sequence
  ATP123
KRYKNRVASRKSRAKFKQLLQHYREVAAAKSSENDRLRLLLKNRTLTLFNVTRNDARAYVSGIQNSVSANRSDPVTLDVLPDSSYLSGANLNLSCHSASPQYSWRINGIPQQHTQVLFIAKITPNNNGTYACFVSNLATGRNNSIVKSITVSASGTSPGLSAAPGSTAPPAHGVTSAPDTRPAPGSTAPPAHGVTSAPDRPALGSTAPPVHNVTSAPPQVLAFGLLLAAATALIYYVDEKAPEFSMQGLKAGVIAVIVVSTVHEILCKLSLEGDHSTPPSAYGSVKPYTNFDAE

SEQ ID NO: 86 - protein, 344 aa, Artificial Sequence
  ATP124
KRYKNRVASRKSRAKFKQLLQHYREVAAAKSSENDRLRLLLKNRTLTLFNVTRNDARAYVSGIQNSVSANRSDPVTLDVLPDSSYLSGANLNLSCHSASPQYSWRINGIPQQHTQVLFIAKITPNNNGTYACFVSNLATGRNNSIVKSITVSASGTSPGLSAAPTLPPAWQPFLKDHRISTFKNWPFLEGSAVKKQFEELTLGEFLKLDRERAPGSTAPPAHGVTSAPDTRPAPGSTAPPAHGVTSAPDRPALGSTAPPVHNVTSAPPQVLAFGLLLAAATALIYYVDEKAPEFSMQGLKAGVIAVIVVSTVHEILCKLSLEGDHSTPPSAYGSVKPYTNFDAE

SEQ ID NO: 87 - protein, 344 aa, Artificial Sequence
  ATP125
KRYKNRVASRKSRAKFKQLLQHYREVAAAKSSENDRLRLLLKNRTLTLFNVTRNDARAYVSGIQNSVSANRSDPVTLDVLPDSSYLSGANLNLSCHSASPQYSWRINGIPQQHTQVLFIAKITPNNNGTYACFVSNLATGRNNSIVKSITVSASGTSPGLSAAPTLPPAWQPFLKDHRISTFKNWPFLEGSAVKKQFEELTLGEFLKLDRERAPGSTAPPAHGVTSAPDTRPAPGSTAPPAHGVTSAPDRPALGSTAPPVHNVTSAPPQVLAFGLLLAAATALIYYVDEKAPEFSMQGLKAGVIAVIVVSTVHEILSKLSLEGDHSTPPSAYGSVKPYTNFDAE

SEQ ID NO: 88 - protein, 397 aa, Artificial Sequence
  ATP127
KRYKNRVASRKSRAKFKQLLQHYREVAAAKSSENDRLRLLLKNRTLTLFNVTRNDARAYVSGIQNSVSANRSDPVTLDVLPDSSYLSGANLNLSCHSASPQYSWRINGIPQQHTQVLFIAKITPNNNGTYACFVSNLATGRNNSIVKSITVSASGTSPGLSAAPTLPPAWQPFLKDHRISTFKNWPFLEGSAVKKQFEELTLGEFLKLDRERAPPQVLAFGLLLAAATALIYYVDEKAPEFSMQGLKAGVIAVIVVAAVARRNERERNRVKLVNLGFQALRQHVPHGGASKKLSKVETLRSAVEYIRALQRLLAEHDAVRNALAGGLRPQAVRPSAPRGPSEGALSPAERELLDFSSWLGGYSTVHEILSKLSLEGDHSTPPSAYGSVKPYTNFDAE

SEQ ID NO: 89 - protein, 353 aa, Artificial Sequence
  ATP128
KRYKNRVASRKSRAKFKQLLQHYREVAAAKSSENDRLRLLLKNRTLTLFNVTRNDARAYVSGIQNSVSANRSDPVTLDVLPDSSYLSGANLNLSCHSASPQYSWRINGIPQQHTQVLFIAKITPNNNGTYACFVSNLATGRNNSIVKSITVSASGTSPGLSAAPTLPPAWQPFLKDHRISTFKNWPFLEGSAVKKQFEELTLGEFLKLDRERAAVARRNERERNRVKLVNLGFQALRQHVPHGGASKKLSKVETLRSAVEYIRALQRLLAEHDAVRNALAGGLRPQAVRPSAPRGPSEGALSPAERELLDFSSWLGGYSTVHEILSKLSLEGDHSTPPSAYGSVKPYTNFDAE

SEQ ID NO: 90 - protein, 358 aa, Artificial Sequence
  ATP129
KRYKNRVASRKSRAKFKQLLQHYREVAAAKSSENDRLRLLLKNRTLTLFNVTRNDARAYVSGIQNSVSANRSDPVTLDVLPDSSYLSGANLNLSCHSASPQYSWRINGIPQQHTQVLFIAKITPNNNGTYACFVSNLATGRNNSIVKSITVSASGTSPGLSAAPTLPPAWQPFLKDHRISTFKNWPFLEGSAVKKQFEELTLGEFLKLDRERAKNKIAAVARRNERERNRVKLVNLGFQALRQHVPHGGASKKLSKVETLRSAVEYIRALQRLLAEHDAVRNALAGGLRPQAVRPSAPRGPSEGALSPAERELLDFSSWLGGYSTVHEILSKLSLEGDHSTPPSAYGSVKPYTNFDAE

SEQ ID NO: 91 - protein, 396 aa, Artificial Sequence
  ATP130
KRYKNRVASRKSRAKFKQLLQHYREVAAAKSSENDRLRLLLKNRTLTLFNVTRNDARAYVSGIQNSVSANRSDPVTLDVLPDSSYLSGANLNLSCHSASPQYSWRINGIPQQHTQVLFIAKITPNNNGTYACFVSNLATGRNNSIVKSITVSASGTSPGLSAAPTLPPAWQPFLKDHRISTFKNWPFLEGSAVKKQFEELTLGEFLKLDRERAKNKIAAVARRNERERNRVKLVNLGFQALRQHVPHGGASKKLSKVETLRSAVEYIRALQRLLAEHDAVRNALAGGLRPQAVRPSAPRGPPGTTPVAASPSRASSSPGRGGSSEPGSPRSAYSSDDSGSEGALSPAERELLDFSSWLGGYSTVHEILSKLSLEGDHSTPPSAYGSVKPYTNFDAE

SEQ ID NO: 92 - protein, 193 aa, Artificial Sequence
  ASCL2
MDGGTLPRSAPPAPPVPVGCAARRRPASPELLRCSRRRRPATAETGGGAAAVARRNERERNRVKLVNLGFQALRQHVPHGGASKKLSKVETLRSAVEYIRALQRLLAEHDAVRNALAGGLRPQAVRPSAPRGPPGTTPVAASPSRASSSPGRGGSSEPGSPRSAYSSDDSGCEGALSPAERELLDFSSWLGGY

SEQ ID NO: 93 - protein, 10 aa, Artificial Sequence
  ASCL2 epitope
SAVEYIRALQ

SEQ ID NO: 94 - protein, 10 aa, Artificial Sequence
  ASCL2 epitope
ERELLDFSSW

SEQ ID NO: 95 - protein, 50 aa, Artificial Sequence
  Survivin fragment
APTLPPAWQPFLKDHRISTFKNWPFLEGSAVKKQFEELTLGEFLKLDRER

SEQ ID NO: 96 - protein, 120 aa, Artificial Sequence
  CEA fragment
NRTLTLFNVTRNDARAYVSGIQNSVSANRSDPVTLDVLPDSSYLSGANLNLSCHSASPQYSWRINGIPQQHTQVLFIAKITPNNNGTYACFVSNLATGRNNSIVKSITVSASGTSPGLSA

SEQ ID NO: 97 - protein, 106 aa, Artificial Sequence
  ASCL2 fragment
AAVARRNERERNRVKLVNLGFQALRQHVPHGGASKKLSKVETLRSAVEYIRALQRLLAEHDAVRNALAGGLRPQAVRPSAPRGPSEGALSPAERELLDFSSWLGGY

SEQ ID NO: 98 - protein, 276 aa, Artificial Sequence
  antigenic cargo of ATP128
NRTLTLFNVTRNDARAYVSGIQNSVSANRSDPVTLDVLPDSSYLSGANLNLSCHSASPQYSWRINGIPQQHTQVLFIAKITPNNNGTYACFVSNLATGRNNSIVKSITVSASGTSPGLSAAPTLPPAWQPFLKDHRISTFKNWPFLEGSAVKKQFEELTLGEFLKLDRERAAVARRNERERNRVKLVNLGFQALRQHVPHGGASKKLSKVETLRSAVEYIRALQRLLAEHDAVRNALAGGLRPQAVRPSAPRGPSEGALSPAERELLDFSSWLGGY